European Patent Application EP 4 261 219 A1, published October 18, 2023. Title: Anti-Allergic Peptide and Use Thereof for Immune Regulation and Anti-Allergy. Applicant: Greenyn Biotechnology Co., Ltd. The sequence listing filed with the application follows.

SEQUENCE LISTING (16 sequences)

SEQ ID NO: 1 - protein, 10 aa, synthetic construct
DLQLAGLIGL

SEQ ID NO: 2 - protein, 9 aa, synthetic construct
NPALQVIKV

SEQ ID NO: 3 - protein, 11 aa, synthetic construct
GLGDAKVALGI

SEQ ID NO: 4 - protein, 9 aa, synthetic construct
EWLLGLLGI

SEQ ID NO: 5 - protein, 10 aa, synthetic construct
DLDVVVALGI

SEQ ID NO: 6 - protein, 11 aa, synthetic construct
VGNSLAAVIIG

SEQ ID NO: 7 - protein, 10 aa, synthetic construct
PMALLAVLGL

SEQ ID NO: 8 - protein, 10 aa, synthetic construct
NKKQAAALGI

SEQ ID NO: 9 - protein, 12 aa, synthetic construct
GVSGGVLAAILG

SEQ ID NO: 10 - protein, 11 aa, synthetic construct
TANAIGLAGLI

SEQ ID NO: 11 - protein, 9 aa, synthetic construct
PPYQGAPLM

SEQ ID NO: 12 - protein, 12 aa, synthetic construct
KIVNQVNHLNPT

SEQ ID NO: 13 - protein, 10 aa, synthetic construct
QTAQALVLIG

SEQ ID NO: 14 - protein, 9 aa, synthetic construct
LVPWSIIGL

SEQ ID NO: 15 - protein, 10 aa, synthetic construct
ADALQLVLAV

SEQ ID NO: 16 - protein, 11 aa, synthetic construct
TRQKALAALGI